European Patent Specification EP 4 105 324 B1, published October 30, 2024. Title: Novel bifunctional pyr operon transcriptional regulator/uracil phosphoribosyltransferase variant and a method for producing IMP using the same. Applicant: CJ CheilJedang Corporation. The sequence listing filed with the application follows.

SEQUENCE LISTING (10 sequences)

SEQ ID NO: 1 - protein, 205 aa, Artificial Sequence
  PyrR_VT
MSGTTVPNDGHEANDAQTNVTQSELLSADDVERTTARIAHQIIEKTALDSPGAARVILLGIPSGGVPLAHRLATKIAEFSGVDIPSGSLDITLYRDDLRNKPHRALQSTSIPAGGIDNAIVVLVDDVLFSGRTIRAALDAIGDIGRPQSIQLAVLVDRGHRQVPIRADYVGKNVPTASNEDIDVLISDIDGRDAVVLTRGITSTQ

SEQ ID NO: 2 - DNA, 618 bp, Artificial Sequence
  pyrR_VT
atgagtggaacaactgtacccaacgacgggcacgaagcaaacgatgcgcagacaaatgtcacgcagtcagaattgctcagtgctgacgacgttgaacgtacaaccgcacgcatcgcgcaccagattattgaaaagacagcattggattcacccggtgctgcgcgagtaattttattgggcatcccttcaggtggcgtgccccttgcacaccggctagcaacaaagattgcagaattttccggtgtggacatccccagtggatccttagatatcacgttgtaccgcgatgatttgcgtaataaaccgcaccgcgctctgcaatcaacatccatcccagccggtggcatcgacaatgccattgtcgttttggtcgatgacgtcctcttttccggccgcaccattcgtgccgctttagacgcgatcggcgatattggtcgcccacagtccattcaattagccgtcttggttgaccgtggccaccgccaggttccaattcgcgctgattatgtaggaaagaacgttccgactgccagcaatgaagacattgatgtccttattagcgatattgacggccgcgacgcggtggtcttgacccgcggcatcacatccacgcaataa

SEQ ID NO: 3 - protein, 205 aa, Artificial Sequence
  PyrR_WT
MSGTTVPNDGHEANDAQTNVTQSELLSADDVERTTARIAHQIIEKTALDSPGAARVILLGIPSGGVPLAHRLATKIAEFSGVDIPSGSLDITLYRDDLRNKPHRALQPTSIPAGGIDNAIVVLVDDVLFSGRTIRAALDAIGDIGRPQSIQLAVLVDRGHRQVPIRADYVGKNVPTASNEDIDVLISDIDGRDAVVLTRGITSTQ

SEQ ID NO: 4 - DNA, 618 bp, Artificial Sequence
  pyrR_WT
atgagtggaacaactgtacccaacgacgggcacgaagcaaacgatgcgcagacaaatgtcacgcagtcagaattgctcagtgctgacgacgttgaacgtacaaccgcacgcatcgcgcaccagattattgaaaagacagcattggattcacccggtgctgcgcgagtaattttattgggcatcccttcaggtggcgtgccccttgcacaccggctagcaacaaagattgcagaattttccggtgtggacatccccagtggatccttagatatcacgttgtaccgcgatgatttgcgtaataaaccgcaccgcgctctgcaaccaacatccatcccagccggtggcatcgacaatgccattgtcgttttggtcgatgacgtcctcttttccggccgcaccattcgtgccgctttagacgcgatcggcgatattggtcgcccacagtccattcaattagccgtcttggttgaccgtggccaccgccaggttccaattcgcgctgattatgtaggaaagaacgttccgactgccagcaatgaagacattgatgtccttattagcgatattgacggccgcgacgcggtggtcttgacccgcggcatcacatccacgcaataa

SEQ ID NO: 5 - DNA, 39 bp, Artificial Sequence
  Primer_1F
gtgaattcgagctcggtaccccaactgtacccaacgacg

SEQ ID NO: 6 - DNA, 33 bp, Artificial Sequence
  Primer_2R
gctgggatggatgttgattgcagagcgcggtgc

SEQ ID NO: 7 - DNA, 33 bp, Artificial Sequence
  Primer_3F
gcaccgcgctctgcaatcaacatccatcccagc

SEQ ID NO: 8 - DNA, 38 bp, Artificial Sequence
  Primer_4R
ggtcgactctagaggatcccccaaacgaggcacgcgtg

SEQ ID NO: 9 - DNA, 18 bp, Artificial Sequence
  Primer_5F
gcgacggtgcgataagtg

SEQ ID NO: 10 - DNA, 17 bp, Artificial Sequence
  Primer_6R
catccgcggacatccac